European Patent Application EP 4 257 134 A2, published October 11, 2023. Title: COMBINING ANTI-HLA-DR OR ANTI-TROP-2 ANTIBODIES WITH MICROTUBULE INHIBITORS, PARP INHIBITORS, BRUTON KINASE INHIBITORS OR PHOSPHOINOSITIDE 3-KINASE INHIBITORS SIGNIFICANTLY IMPROVES THERAPEUTIC OUTCOME IN CANCER. Applicant: IMMUNOMEDICS, INC. The sequence listing filed with the application follows.

SEQUENCE LISTING (161 sequences)

SEQ ID NO: 1 - protein, 44 aa, synthetic construct
  REGION 1..44: note = Description of Artificial Sequence: Synthetic polypeptide
SHIQIPPGLTELLQGYTVEVLRQQPPDLVEFAVEYFTRLREARA

SEQ ID NO: 2 - protein, 45 aa, synthetic construct
  REGION 1..45: note = Description of Artificial Sequence: Synthetic polypeptide
CGHIQIPPGLTELLQGYTVEVLRQQPPDLVEFAVEYFTRLREARA

SEQ ID NO: 3 - protein, 17 aa, synthetic construct
  REGION 1..17: note = Description of Artificial Sequence: Synthetic peptide
QIEYLAKQIVDNAIQQA

SEQ ID NO: 4 - protein, 21 aa, synthetic construct
  REGION 1..21: note = Description of Artificial Sequence: Synthetic peptide
CGQIEYLAKQIVDNAIQQAGC

SEQ ID NO: 5 - protein, 50 aa, synthetic construct
  REGION 1..50: note = Description of Artificial Sequence: Synthetic polypeptide
SLRECELYVQKHNIQALLKDSIVQLCTARPERPMAFLREYFERLEKEEAK

SEQ ID NO: 6 - protein, 55 aa, synthetic construct
  REGION 1..55: note = Description of Artificial Sequence: Synthetic polypeptide
MSCGGSLRECELYVQKHNIQALLKDSIVQLCTARPERPMAFLREYFERLEKEEAK

SEQ ID NO: 7 - protein, 23 aa, synthetic construct
  REGION 1..23: note = Description of Artificial Sequence: Synthetic peptide
CGFEELAWKIAKMIWSDVFQQGC

SEQ ID NO: 8 - protein, 51 aa, synthetic construct
  REGION 1..51: note = Description of Artificial Sequence: Synthetic polypeptide
SLRECELYVQKHNIQALLKDVSIVQLCTARPERPMAFLREYFEKLEKEEAK

SEQ ID NO: 9 - protein, 54 aa, synthetic construct
  REGION 1..54: note = Description of Artificial Sequence: Synthetic polypeptide
SLKGCELYVQLHGIQQVLKDCIVHLCISKPERPMKFLREHFEKLEKEENRQILA

SEQ ID NO: 10 - protein, 44 aa, synthetic construct
  REGION 1..44: note = Description of Artificial Sequence: Synthetic polypeptide
SHIQIPPGLTELLQGYTVEVGQQPPDLVDFAVEYFTRLREARRQ

SEQ ID NO: 11 - protein, 44 aa, synthetic construct
  REGION 1..44: note = Description of Artificial Sequence: Synthetic polypeptide
SIEIPAGLTELLQGFTVEVLRHQPADLLEFALQHFTRLQQENER

SEQ ID NO: 12 - protein, 44 aa, synthetic construct
  REGION 1..44: note = Description of Artificial Sequence: Synthetic polypeptide
THIQIPPGLTELLQGYTVEVLRQQPPDLVEFAVEYFTRLREARA

SEQ ID NO: 13 - protein, 44 aa, synthetic construct
  REGION 1..44: note = Description of Artificial Sequence: Synthetic polypeptide
SKIQIPPGLTELLQGYTVEVLRQQPPDLVEFAVEYFTRLREARA

SEQ ID NO: 14 - protein, 44 aa, synthetic construct
  REGION 1..44: note = Description of Artificial Sequence: Synthetic polypeptide
SRIQIPPGLTELLQGYTVEVLRQQPPDLVEFAVEYFTRLREARA

SEQ ID NO: 15 - protein, 44 aa, synthetic construct
  REGION 1..44: note = Description of Artificial Sequence: Synthetic polypeptide
SHINIPPGLTELLQGYTVEVLRQQPPDLVEFAVEYFTRLREARA

SEQ ID NO: 16 - protein, 44 aa, synthetic construct
  REGION 1..44: note = Description of Artificial Sequence: Synthetic polypeptide
SHIQIPPALTELLQGYTVEVLRQQPPDLVEFAVEYFTRLREARA

SEQ ID NO: 17 - protein, 44 aa, synthetic construct
  REGION 1..44: note = Description of Artificial Sequence: Synthetic polypeptide
SHIQIPPGLSELLQGYTVEVLRQQPPDLVEFAVEYFTRLREARA

SEQ ID NO: 18 - protein, 44 aa, synthetic construct
  REGION 1..44: note = Description of Artificial Sequence: Synthetic polypeptide
SHIQIPPGLTDLLQGYTVEVLRQQPPDLVEFAVEYFTRLREARA

SEQ ID NO: 19 - protein, 44 aa, synthetic construct
  REGION 1..44: note = Description of Artificial Sequence: Synthetic polypeptide
SHIQIPPGLTELLNGYTVEVLRQQPPDLVEFAVEYFTRLREARA

SEQ ID NO: 20 - protein, 44 aa, synthetic construct
  REGION 1..44: note = Description of Artificial Sequence: Synthetic polypeptide
SHIQIPPGLTELLQAYTVEVLRQQPPDLVEFAVEYFTRLREARA

SEQ ID NO: 21 - protein, 44 aa, synthetic construct
  REGION 1..44: note = Description of Artificial Sequence: Synthetic polypeptide
SHIQIPPGLTELLQGYSVEVLRQQPPDLVEFAVEYFTRLREARA

SEQ ID NO: 22 - protein, 44 aa, synthetic construct
  REGION 1..44: note = Description of Artificial Sequence: Synthetic polypeptide
SHIQIPPGLTELLQGYTVDVLRQQPPDLVEFAVEYFTRLREARA

SEQ ID NO: 23 - protein, 44 aa, synthetic construct
  REGION 1..44: note = Description of Artificial Sequence: Synthetic polypeptide
SHIQIPPGLTELLQGYTVEVLKQQPPDLVEFAVEYFTRLREARA

SEQ ID NO: 24 - protein, 44 aa, synthetic construct
  REGION 1..44: note = Description of Artificial Sequence: Synthetic polypeptide
SHIQIPPGLTELLQGYTVEVLRNQPPDLVEFAVEYFTRLREARA

SEQ ID NO: 25 - protein, 44 aa, synthetic construct
  REGION 1..44: note = Description of Artificial Sequence: Synthetic polypeptide
SHIQIPPGLTELLQGYTVEVLRQNPPDLVEFAVEYFTRLREARA

SEQ ID NO: 26 - protein, 44 aa, synthetic construct
  REGION 1..44: note = Description of Artificial Sequence: Synthetic polypeptide
SHIQIPPGLTELLQGYTVEVLRQQPPELVEFAVEYFTRLREARA

SEQ ID NO: 27 - protein, 44 aa, synthetic construct
  REGION 1..44: note = Description of Artificial Sequence: Synthetic polypeptide
SHIQIPPGLTELLQGYTVEVLRQQPPDLVDFAVEYFTRLREARA

SEQ ID NO: 28 - protein, 44 aa, synthetic construct
  REGION 1..44: note = Description of Artificial Sequence: Synthetic polypeptide
SHIQIPPGLTELLQGYTVEVLRQQPPDLVEFLVEYFTRLREARA

SEQ ID NO: 29 - protein, 44 aa, synthetic construct
  REGION 1..44: note = Description of Artificial Sequence: Synthetic polypeptide
SHIQIPPGLTELLQGYTVEVLRQQPPDLVEFIVEYFTRLREARA

SEQ ID NO: 30 - protein, 44 aa, synthetic construct
  REGION 1..44: note = Description of Artificial Sequence: Synthetic polypeptide
SHIQIPPGLTELLQGYTVEVLRQQPPDLVEFVVEYFTRLREARA

SEQ ID NO: 31 - protein, 44 aa, synthetic construct
  REGION 1..44: note = Description of Artificial Sequence: Synthetic polypeptide
SHIQIPPGLTELLQGYTVEVLRQQPPDLVEFAVDYFTRLREARA

SEQ ID NO: 32 - protein, 17 aa, synthetic construct
  REGION 1..17: note = Description of Artificial Sequence: Synthetic peptide
NIEYLAKQIVDNAIQQA

SEQ ID NO: 33 - protein, 17 aa, synthetic construct
  REGION 1..17: note = Description of Artificial Sequence: Synthetic peptide
QLEYLAKQIVDNAIQQA

SEQ ID NO: 34 - protein, 17 aa, synthetic construct
  REGION 1..17: note = Description of Artificial Sequence: Synthetic peptide
QVEYLAKQIVDNAIQQA

SEQ ID NO: 35 - protein, 17 aa, synthetic construct
  REGION 1..17: note = Description of Artificial Sequence: Synthetic peptide
QIDYLAKQIVDNAIQQA

SEQ ID NO: 36 - protein, 17 aa, synthetic construct
  REGION 1..17: note = Description of Artificial Sequence: Synthetic peptide
QIEFLAKQIVDNAIQQA

SEQ ID NO: 37 - protein, 17 aa, synthetic construct
  REGION 1..17: note = Description of Artificial Sequence: Synthetic peptide
QIETLAKQIVDNAIQQA

SEQ ID NO: 38 - protein, 17 aa, synthetic construct
  REGION 1..17: note = Description of Artificial Sequence: Synthetic peptide
QIESLAKQIVDNAIQQA

SEQ ID NO: 39 - protein, 17 aa, synthetic construct
  REGION 1..17: note = Description of Artificial Sequence: Synthetic peptide
QIEYIAKQIVDNAIQQA

SEQ ID NO: 40 - protein, 17 aa, synthetic construct
  REGION 1..17: note = Description of Artificial Sequence: Synthetic peptide
QIEYVAKQIVDNAIQQA

SEQ ID NO: 41 - protein, 17 aa, synthetic construct
  REGION 1..17: note = Description of Artificial Sequence: Synthetic peptide
QIEYLARQIVDNAIQQA

SEQ ID NO: 42 - protein, 17 aa, synthetic construct
  REGION 1..17: note = Description of Artificial Sequence: Synthetic peptide
QIEYLAKNIVDNAIQQA

SEQ ID NO: 43 - protein, 17 aa, synthetic construct
  REGION 1..17: note = Description of Artificial Sequence: Synthetic peptide
QIEYLAKQIVENAIQQA

SEQ ID NO: 44 - protein, 17 aa, synthetic construct
  REGION 1..17: note = Description of Artificial Sequence: Synthetic peptide
QIEYLAKQIVDQAIQQA

SEQ ID NO: 45 - protein, 17 aa, synthetic construct
  REGION 1..17: note = Description of Artificial Sequence: Synthetic peptide
QIEYLAKQIVDNAINQA

SEQ ID NO: 46 - protein, 17 aa, synthetic construct
  REGION 1..17: note = Description of Artificial Sequence: Synthetic peptide
QIEYLAKQIVDNAIQNA

SEQ ID NO: 47 - protein, 17 aa, synthetic construct
  REGION 1..17: note = Description of Artificial Sequence: Synthetic peptide
QIEYLAKQIVDNAIQQL

SEQ ID NO: 48 - protein, 17 aa, synthetic construct
  REGION 1..17: note = Description of Artificial Sequence: Synthetic peptide
QIEYLAKQIVDNAIQQI

SEQ ID NO: 49 - protein, 17 aa, synthetic construct
  REGION 1..17: note = Description of Artificial Sequence: Synthetic peptide
QIEYLAKQIVDNAIQQV

SEQ ID NO: 50 - protein, 17 aa, synthetic construct
  REGION 1..17: note = Description of Artificial Sequence: Synthetic peptide
QIEYVAKQIVDYAIHQA

SEQ ID NO: 51 - protein, 17 aa, synthetic construct
  REGION 1..17: note = Description of Artificial Sequence: Synthetic peptide
QIEYKAKQIVDHAIHQA

SEQ ID NO: 52 - protein, 17 aa, synthetic construct
  REGION 1..17: note = Description of Artificial Sequence: Synthetic peptide
QIEYHAKQIVDHAIHQA

SEQ ID NO: 53 - protein, 17 aa, synthetic construct
  REGION 1..17: note = Description of Artificial Sequence: Synthetic peptide
QIEYVAKQIVDHAIHQA

SEQ ID NO: 54 - protein, 18 aa, synthetic construct
  REGION 1..18: note = Description of Artificial Sequence: Synthetic peptide
PLEYQAGLLVQNAIQQAI

SEQ ID NO: 55 - protein, 18 aa, synthetic construct
  REGION 1..18: note = Description of Artificial Sequence: Synthetic peptide
LLIETASSLVKNAIQLSI

SEQ ID NO: 56 - protein, 18 aa, synthetic construct
  REGION 1..18: note = Description of Artificial Sequence: Synthetic peptide
LIEEAASRIVDAVIEQVK

SEQ ID NO: 57 - protein, 18 aa, synthetic construct
  REGION 1..18: note = Description of Artificial Sequence: Synthetic peptide
ALYQFADRFSELVISEAL

SEQ ID NO: 58 - protein, 17 aa, synthetic construct
  REGION 1..17: note = Description of Artificial Sequence: Synthetic peptide
LEQVANQLADQIIKEAT

SEQ ID NO: 59 - protein, 17 aa, synthetic construct
  REGION 1..17: note = Description of Artificial Sequence: Synthetic peptide
FEELAWKIAKMIWSDVF

SEQ ID NO: 60 - protein, 18 aa, synthetic construct
  REGION 1..18: note = Description of Artificial Sequence: Synthetic peptide
ELVRLSKRLVENAVLKAV

SEQ ID NO: 61 - protein, 18 aa, synthetic construct
  REGION 1..18: note = Description of Artificial Sequence: Synthetic peptide
TAEEVSARIVQVVTAEAV

SEQ ID NO: 62 - protein, 18 aa, synthetic construct
  REGION 1..18: note = Description of Artificial Sequence: Synthetic peptide
QIKQAAFQLISQVILEAT

SEQ ID NO: 63 - protein, 16 aa, synthetic construct
  REGION 1..16: note = Description of Artificial Sequence: Synthetic peptide
LAWKIAKMIVSDVMQQ

SEQ ID NO: 64 - protein, 24 aa, synthetic construct
  REGION 1..24: note = Description of Artificial Sequence: Synthetic peptide
DLIEEAASRIVDAVIEQVKAAGAY

SEQ ID NO: 65 - protein, 18 aa, synthetic construct
  REGION 1..18: note = Description of Artificial Sequence: Synthetic peptide
LEQYANQLADQIIKEATE

SEQ ID NO: 66 - protein, 20 aa, synthetic construct
  REGION 1..20: note = Description of Artificial Sequence: Synthetic peptide
FEELAWKIAKMIWSDVFQQC

SEQ ID NO: 67 - protein, 17 aa, synthetic construct
  REGION 1..17: note = Description of Artificial Sequence: Synthetic peptide
QIEYLAKQIPDNAIQQA

SEQ ID NO: 68 - protein, 25 aa, synthetic construct
  REGION 1..25: note = Description of Artificial Sequence: Synthetic peptide
KGADLIEEAASRIVDAVIEQVKAAG

SEQ ID NO: 69 - protein, 25 aa, synthetic construct
  REGION 1..25: note = Description of Artificial Sequence: Synthetic peptide
KGADLIEEAASRIPDAPIEQVKAAG

SEQ ID NO: 70 - protein, 25 aa, synthetic construct
  REGION 1..25: note = Description of Artificial Sequence: Synthetic peptide
PEDAELVRLSKRLVENAVLKAVQQY

SEQ ID NO: 71 - protein, 25 aa, synthetic construct
  REGION 1..25: note = Description of Artificial Sequence: Synthetic peptide
PEDAELVRTSKRLVENAVLKAVQQY

SEQ ID NO: 72 - protein, 25 aa, synthetic construct
  REGION 1..25: note = Description of Artificial Sequence: Synthetic peptide
PEDAELVRLSKRDVENAVLKAVQQY

SEQ ID NO: 73 - protein, 25 aa, synthetic construct
  REGION 1..25: note = Description of Artificial Sequence: Synthetic peptide
PEDAELVRLSKRLPENAVLKAVQQY

SEQ ID NO: 74 - protein, 25 aa, synthetic construct
  REGION 1..25: note = Description of Artificial Sequence: Synthetic peptide
PEDAELVRLSKRLPENAPLKAVQQY

SEQ ID NO: 75 - protein, 25 aa, synthetic construct
  REGION 1..25: note = Description of Artificial Sequence: Synthetic peptide
PEDAELVRLSKRLVENAVEKAVQQY

SEQ ID NO: 76 - protein, 25 aa, synthetic construct
  REGION 1..25: note = Description of Artificial Sequence: Synthetic peptide
EEGLDRNEEIKRAAFQIISQVISEA

SEQ ID NO: 77 - protein, 25 aa, synthetic construct
  REGION 1..25: note = Description of Artificial Sequence: Synthetic peptide
LVDDPLEYQAGLLVQNAIQQAIAEQ

SEQ ID NO: 78 - protein, 25 aa, synthetic construct
  REGION 1..25: note = Description of Artificial Sequence: Synthetic peptide
QYETLLIETASSLVKNAIQLSIEQL

SEQ ID NO: 79 - protein, 25 aa, synthetic construct
  REGION 1..25: note = Description of Artificial Sequence: Synthetic peptide
LEKQYQEQLEEEVAKVIVSMSIAFA

SEQ ID NO: 80 - protein, 25 aa, synthetic construct
  REGION 1..25: note = Description of Artificial Sequence: Synthetic peptide
NTDEAQEELAWKIAKMIVSDIMQQA

SEQ ID NO: 81 - protein, 25 aa, synthetic construct
  REGION 1..25: note = Description of Artificial Sequence: Synthetic peptide
VNLDKKAVLAEKIVAEAIEKAEREL

SEQ ID NO: 82 - protein, 25 aa, synthetic construct
  REGION 1..25: note = Description of Artificial Sequence: Synthetic peptide
NGILELETKSSKLVQNIIQTAVDQF

SEQ ID NO: 83 - protein, 25 aa, synthetic construct
  REGION 1..25: note = Description of Artificial Sequence: Synthetic peptide
TQDKNYEDELTQVALALVEDVINYA

SEQ ID NO: 84 - protein, 25 aa, synthetic construct
  REGION 1..25: note = Description of Artificial Sequence: Synthetic peptide
ETSAKDNINIEEAARFLVEKILVNH

SEQ ID NO: 85 - protein, 330 aa, synthetic construct
  REGION 1..330: note = Description of Artificial Sequence: Synthetic polypeptide
ASTKGPSVFPLAPSSKSTSGGTAALGCLVKDYFPEPVTVSWNSGALTSGVHTFPAVLQSSGLYSLSSVVTVPSSSLGTQTYICNVNHKPSNTKVDKKAEPKSCDKTHTCPPCPAPELLGGPSVFLFPPKPKDTLMISRTPEVTCVVVDVSHEDPEVKFNWYVDGVEVHNAKTKPREEQYNSTYRVVSVLTVLHQDWLNGKEYKCKVSNKALPAPIEKTISKAKGQPREPQVYTLPPSRDELTKNQVSLTCLVKGFYPSDIAVEWESNGQPENNYKTTPPVLDSDGSFFLYSKLTVDKSRWQQGNVFSCSVMHEALHNHYTQKSLSLSPGK

SEQ ID NO: 86 - protein, 330 aa, synthetic construct
  REGION 1..330: note = Description of Artificial Sequence: Synthetic polypeptide
ASTKGPSVFPLAPSSKSTSGGTAALGCLVKDYFPEPVTVSWNSGALTSGVHTFPAVLQSSGLYSLSSVVTVPSSSLGTQTYICNVNHKPSNTKVDKRVEPKSCDKTHTCPPCPAPELLGGPSVFLFPPKPKDTLMISRTPEVTCVVVDVSHEDPEVKFNWYVDGVEVHNAKTKPREEQYNSTYRVVSVLTVLHQDWLNGKEYKCKVSNKALPAPIEKTISKAKGQPREPQVYTLPPSREEMTKNQVSLTCLVKGFYPSDIAVEWESNGQPENNYKTTPPVLDSDGSFFLYSKLTVDKSRWQQGNVFSCSVMHEALHNHYTQKSLSLSPGK

SEQ ID NO: 87 - protein, 44 aa, synthetic construct
  REGION 1..44: note = Description of Artificial Sequence: Synthetic consensus polypeptide
  VARIANT 1: note = MOD_RES - Ser or Thr
  VARIANT 2: note = MOD_RES - His, Lys or Arg
  VARIANT 4: note = MOD_RES - Gln or Asn
  VARIANT 8: note = MOD_RES - Gly or Ala
  VARIANT 10: note = MOD_RES - Thr or Ser
  VARIANT 11: note = MOD_RES - Glu or Asp
  VARIANT 14: note = MOD_RES - Gln or Asn
  VARIANT 15: note = MOD_RES - Gly or Ala
  VARIANT 17: note = MOD_RES - Thr or Ser
  VARIANT 19: note = MOD_RES - Glu or Asp
  VARIANT 22: note = MOD_RES - Arg or Lys
  VARIANT 23..24: note = MOD_RES - Asn or Gln
  VARIANT 27: note = MOD_RES - Asp or Glu
  VARIANT 30: note = MOD_RES - Glu or Asp
  VARIANT 32: note = MOD_RES - Ala, Leu, Ile or Val
  VARIANT 34: note = MOD_RES - Glu or Asp
  VARIANT 37: note = MOD_RES - Thr or Ser
  VARIANT 38: note = MOD_RES - Arg or Lys
  VARIANT 40: note = MOD_RES - Arg or Lys
  VARIANT 41: note = MOD_RES - Glu or Asp
  VARIANT 42: note = MOD_RES - Ala, Leu, Ile or Val
  VARIANT 43: note = MOD_RES - Arg or Lys
  VARIANT 44: note = MOD_RES - Ala, Leu, Ile or Val
XXIXIPPXLXXLLXXYXVXVLXXXPPXLVXFXVXYFXXLXXXXX

SEQ ID NO: 88 - protein, 17 aa, synthetic construct
  REGION 1..17: note = Description of Artificial Sequence: Synthetic consensus peptide
  VARIANT 1: note = MOD_RES - Gln or Asn
  VARIANT 2: note = MOD_RES - Ile, Leu or Val
  VARIANT 3: note = MOD_RES - Glu or Asp
  VARIANT 4: note = MOD_RES - Tyr, Phe, Thr or Ser
  VARIANT 5: note = MOD_RES - Leu, Ile or Val
  VARIANT 7: note = MOD_RES - Lys or Arg
  VARIANT 8: note = MOD_RES - Gln or Asn
  VARIANT 11: note = MOD_RES - Asp or Glu
  VARIANT 12: note = MOD_RES - Asn or Gln
  VARIANT 15..16: note = MOD_RES - Gln or Asn
  VARIANT 17: note = MOD_RES - Ala, Leu, Ile or Val
XXXXXAXXIVXXAIXXX

SEQ ID NO: 89 - protein, 44 aa, synthetic construct
  REGION 1..44: note = Description of Artificial Sequence: Synthetic consensus polypeptide
  VARIANT 1: note = MOD_RES - Ser or Thr
  VARIANT 4: note = MOD_RES - Gln or Asn
  VARIANT 10: note = MOD_RES - Thr or Ser
  VARIANT 18: note = MOD_RES - Val, Ile, Leu or Ala
  VARIANT 23: note = MOD_RES - Gln or Asn
  VARIANT 33: note = MOD_RES - Val, Ile, Leu or Ala
  VARIANT 34: note = MOD_RES - Glu or Asp
  VARIANT 37: note = MOD_RES - Thr or Ser
  VARIANT 38: note = MOD_RES - Arg or Lys
  VARIANT 40: note = MOD_RES - Arg or Lys
  VARIANT 42: note = MOD_RES - Ala, Leu, Ile or Val
  VARIANT 44: note = MOD_RES - Ala, Leu, Ile or Val
XHIXIPPGLXELLQGYTXEVLRXQPPDLVEFAXXYFXXLXEXRX

SEQ ID NO: 90 - protein, 11 aa, synthetic construct
  REGION 1..11: note = Description of Artificial Sequence: Synthetic peptide
KASQDVSIAVA

SEQ ID NO: 91 - protein, 7 aa, synthetic construct
  REGION 1..7: note = Description of Artificial Sequence: Synthetic peptide
SASYRYT

SEQ ID NO: 92 - protein, 9 aa, synthetic construct
  REGION 1..9: note = Description of Artificial Sequence: Synthetic peptide
QQHYITPLT

SEQ ID NO: 93 - protein, 5 aa, synthetic construct
  REGION 1..5: note = Description of Artificial Sequence: Synthetic peptide
NYGMN

SEQ ID NO: 94 - protein, 17 aa, synthetic construct
  REGION 1..17: note = Description of Artificial Sequence: Synthetic peptide
WINTYTGEPTYTDDFKG

SEQ ID NO: 95 - protein, 12 aa, synthetic construct
  REGION 1..12: note = Description of Artificial Sequence: Synthetic peptide
GGFGSSYWYFDV

SEQ ID NO: 96 - protein, 11 aa, synthetic construct
  REGION 1..11: note = Description of Artificial Sequence: Synthetic peptide
KASQDVGTSVA

SEQ ID NO: 97 - protein, 7 aa, synthetic construct
  REGION 1..7: note = Description of Artificial Sequence: Synthetic peptide
WTSTRHT

SEQ ID NO: 98 - protein, 8 aa, synthetic construct
  REGION 1..8: note = Description of Artificial Sequence: Synthetic peptide
QQYSLYRS

SEQ ID NO: 99 - protein, 5 aa, synthetic construct
  REGION 1..5: note = Description of Artificial Sequence: Synthetic peptide
TYWMS

SEQ ID NO: 100 - protein, 17 aa, synthetic construct
  REGION 1..17: note = Description of Artificial Sequence: Synthetic peptide
EIHPDSSTINYAPSLKD

SEQ ID NO: 101 - protein, 10 aa, synthetic construct
  REGION 1..10: note = Description of Artificial Sequence: Synthetic peptide
LYFGFPWFAY

SEQ ID NO: 102 - protein, 16 aa, synthetic construct
  REGION 1..16: note = Description of Artificial Sequence: Synthetic peptide
RSSQSIVHSNGNTYLE

SEQ ID NO: 103 - protein, 7 aa, synthetic construct
  REGION 1..7: note = Description of Artificial Sequence: Synthetic peptide
KVSNRFS

SEQ ID NO: 104 - protein, 9 aa, synthetic construct
  REGION 1..9: note = Description of Artificial Sequence: Synthetic peptide
FQGSHVPPT

SEQ ID NO: 105 - protein, 5 aa, synthetic construct
  REGION 1..5: note = Description of Artificial Sequence: Synthetic peptide
NYGMN

SEQ ID NO: 106 - protein, 17 aa, synthetic construct
  REGION 1..17: note = Description of Artificial Sequence: Synthetic peptide
WINTYTGEPTYADDFKG

SEQ ID NO: 107 - protein, 12 aa, synthetic construct
  REGION 1..12: note = Description of Artificial Sequence: Synthetic peptide
KGWMDFNSSLDY

SEQ ID NO: 108 - protein, 10 aa, synthetic construct
  REGION 1..10: note = Description of Artificial Sequence: Synthetic peptide
SASSRVSYIH

SEQ ID NO: 109 - protein, 7 aa, synthetic construct
  REGION 1..7: note = Description of Artificial Sequence: Synthetic peptide
GTSTLAS

SEQ ID NO: 110 - protein, 9 aa, synthetic construct
  REGION 1..9: note = Description of Artificial Sequence: Synthetic peptide
QQWSYNPPT

SEQ ID NO: 111 - protein, 5 aa, synthetic construct
  REGION 1..5: note = Description of Artificial Sequence: Synthetic peptide
DYYMS

SEQ ID NO: 112 - protein, 19 aa, synthetic construct
  REGION 1..19: note = Description of Artificial Sequence: Synthetic peptide
FIANKANGHTTDYSPSVKG

SEQ ID NO: 113 - protein, 10 aa, synthetic construct
  REGION 1..10: note = Description of Artificial Sequence: Synthetic peptide
DMGIRWNFDV

SEQ ID NO: 114 - protein, 16 aa, synthetic construct
  REGION 1..16: note = Description of Artificial Sequence: Synthetic peptide
RSSQSLVHRNGNTYLH

SEQ ID NO: 115 - protein, 7 aa, synthetic construct
  REGION 1..7: note = Description of Artificial Sequence: Synthetic peptide
TVSNRFS

SEQ ID NO: 116 - protein, 9 aa, synthetic construct
  REGION 1..9: note = Description of Artificial Sequence: Synthetic peptide
SQSSHVPPT

SEQ ID NO: 117 - protein, 5 aa, synthetic construct
  REGION 1..5: note = Description of Artificial Sequence: Synthetic peptide
NYGVN

SEQ ID NO: 118 - protein, 17 aa, synthetic construct
  REGION 1..17: note = Description of Artificial Sequence: Synthetic peptide
WINPNTGEPTFDDDFKG

SEQ ID NO: 119 - protein, 11 aa, synthetic construct
  REGION 1..11: note = Description of Artificial Sequence: Synthetic peptide
SRGKNEAWFAY

SEQ ID NO: 120 - protein, 16 aa, synthetic construct
  REGION 1..16: note = Description of Artificial Sequence: Synthetic peptide
KSSQSVLYSANHKYLA

SEQ ID NO: 121 - protein, 7 aa, synthetic construct
  REGION 1..7: note = Description of Artificial Sequence: Synthetic peptide
WASTRES

SEQ ID NO: 122 - protein, 9 aa, synthetic construct
  REGION 1..9: note = Description of Artificial Sequence: Synthetic peptide
HQYLSSWTF

SEQ ID NO: 123 - protein, 5 aa, synthetic construct
  REGION 1..5: note = Description of Artificial Sequence: Synthetic peptide
SYWLH

SEQ ID NO: 124 - protein, 17 aa, synthetic construct
  REGION 1..17: note = Description of Artificial Sequence: Synthetic peptide
YINPRNDYTEYNQNFKD

SEQ ID NO: 125 - protein, 7 aa, synthetic construct
  REGION 1..7: note = Description of Artificial Sequence: Synthetic peptide
RDITTFY

SEQ ID NO: 126 - protein, 16 aa, synthetic construct
  REGION 1..16: note = Description of Artificial Sequence: Synthetic peptide
RSSQSIVHSNGNTYLE

SEQ ID NO: 127 - protein, 7 aa, synthetic construct
  REGION 1..7: note = Description of Artificial Sequence: Synthetic peptide
KVSNRFS

SEQ ID NO: 128 - protein, 9 aa, synthetic construct
  REGION 1..9: note = Description of Artificial Sequence: Synthetic peptide
FQGSRVPYT

SEQ ID NO: 129 - protein, 5 aa, synthetic construct
  REGION 1..5: note = Description of Artificial Sequence: Synthetic peptide
EYVIT

SEQ ID NO: 130 - protein, 16 aa, synthetic construct
  REGION 1..16: note = Description of Artificial Sequence: Synthetic peptide
EIYPGSGSTSYNEKFK

SEQ ID NO: 131 - skipped

SEQ ID NO: 132 - protein, 12 aa, synthetic construct
  REGION 1..12: note = Description of Artificial Sequence: Synthetic peptide
SASSSVSSSYLY

SEQ ID NO: 133 - protein, 7 aa, synthetic construct
  REGION 1..7: note = Description of Artificial Sequence: Synthetic peptide
STSNLAS

SEQ ID NO: 134 - protein, 9 aa, synthetic construct
  REGION 1..9: note = Description of Artificial Sequence: Synthetic peptide
HQWNRYPYT

SEQ ID NO: 135 - protein, 5 aa, synthetic construct
  REGION 1..5: note = Description of Artificial Sequence: Synthetic peptide
SYVLH

SEQ ID NO: 136 - protein, 17 aa, synthetic construct
  REGION 1..17: note = Description of Artificial Sequence: Synthetic peptide
YINPYNDGTQYNEKFKG

SEQ ID NO: 137 - protein, 10 aa, synthetic construct
  REGION 1..10: note = Description of Artificial Sequence: Synthetic peptide
GFGGSYGFAY

SEQ ID NO: 138 - protein, 5 aa, synthetic construct
  REGION 1..5: note = Description of Artificial Sequence: Synthetic peptide
SYVIH

SEQ ID NO: 139 - protein, 17 aa, synthetic construct
  REGION 1..17: note = Description of Artificial Sequence: Synthetic peptide
YIHPYNGGTKYNEKFKG

SEQ ID NO: 140 - protein, 9 aa, synthetic construct
  REGION 1..9: note = Description of Artificial Sequence: Synthetic peptide
SGGGDPFAY

SEQ ID NO: 141 - protein, 11 aa, synthetic construct
  REGION 1..11: note = Description of Artificial Sequence: Synthetic peptide
KASQDINKYIG

SEQ ID NO: 142 - protein, 7 aa, synthetic construct
  REGION 1..7: note = Description of Artificial Sequence: Synthetic peptide
YTSALLP

SEQ ID NO: 143 - protein, 8 aa, synthetic construct
  REGION 1..8: note = Description of Artificial Sequence: Synthetic peptide
LQYDDLWT

SEQ ID NO: 144 - protein, 5 aa, synthetic construct
  REGION 1..5: note = Description of Artificial Sequence: Synthetic peptide
NYGMN

SEQ ID NO: 145 - protein, 17 aa, synthetic construct
  REGION 1..17: note = Description of Artificial Sequence: Synthetic peptide
WINTYTREPTYADDFKG

SEQ ID NO: 146 - protein, 12 aa, synthetic construct
  REGION 1..12: note = Description of Artificial Sequence: Synthetic peptide
DITAVVPTGFDY

SEQ ID NO: 147 - protein, 11 aa, synthetic construct
  REGION 1..11: note = Description of Artificial Sequence: Synthetic peptide
RASENIYSNLA

SEQ ID NO: 148 - protein, 7 aa, synthetic construct
  REGION 1..7: note = Description of Artificial Sequence: Synthetic peptide
AASNLAD

SEQ ID NO: 149 - protein, 9 aa, synthetic construct
  REGION 1..9: note = Description of Artificial Sequence: Synthetic peptide
QHFWTTPWA

SEQ ID NO: 150 - protein, 10 aa, synthetic construct
  REGION 1..10: note = Description of Artificial Sequence: Synthetic peptide
RASSSVSYIH

SEQ ID NO: 151 - protein, 7 aa, synthetic construct
  REGION 1..7: note = Description of Artificial Sequence: Synthetic peptide
ATSNLAS

SEQ ID NO: 152 - protein, 9 aa, synthetic construct
  REGION 1..9: note = Description of Artificial Sequence: Synthetic peptide
QQWTSNPPT

SEQ ID NO: 153 - protein, 5 aa, synthetic construct
  REGION 1..5: note = Description of Artificial Sequence: Synthetic peptide
SYNMH

SEQ ID NO: 154 - protein, 17 aa, synthetic construct
  REGION 1..17: note = Description of Artificial Sequence: Synthetic peptide
AIYPGNGDTSYNQKFKG

SEQ ID NO: 155 - protein, 12 aa, synthetic construct
  REGION 1..12: note = Description of Artificial Sequence: Synthetic peptide
STYYGGDWYFDV

SEQ ID NO: 156 - protein, 15 aa, synthetic construct
  REGION 1..15: note = Description of Artificial Sequence: Synthetic peptide
KASQSVDYDGDSYLN

SEQ ID NO: 157 - protein, 7 aa, synthetic construct
  REGION 1..7: note = Description of Artificial Sequence: Synthetic peptide
DASNLVS

SEQ ID NO: 158 - protein, 9 aa, synthetic construct
  REGION 1..9: note = Description of Artificial Sequence: Synthetic peptide
QQSTEDPWT

SEQ ID NO: 159 - protein, 5 aa, synthetic construct
  REGION 1..5: note = Description of Artificial Sequence: Synthetic peptide
SYWMN

SEQ ID NO: 160 - protein, 17 aa, synthetic construct
  REGION 1..17: note = Description of Artificial Sequence: Synthetic peptide
QIWPGDGDTNYNGKFKG

SEQ ID NO: 161 - protein, 15 aa, synthetic construct
  REGION 1..15: note = Description of Artificial Sequence: Synthetic peptide
RETTTVGRYYYAMDY